European Patent Application EP 4 666 998 A1, published December 24, 2025. Title: COMPOSITION COMPRENANT UN POLYMERE BIOCOMPATIBLE ET DES VESICULES EXTRACELLULAIRES ET PROCEDE DE PREPARATION. Applicant: Organes Tissus Régénération Réparation Remplacement. The sequence listing filed with the application follows.

SEQUENCE LISTING (31 sequences)

SEQ ID NO: 1 - protein, 11 aa, synthetic construct
RVRAQHRERVT

SEQ ID NO: 2 - protein, 10 aa, synthetic construct
SVRLRGLRPL

SEQ ID NO: 3 - protein, 10 aa, synthetic construct
ARGYRLEWRR

SEQ ID NO: 4 - protein, 12 aa, synthetic construct
HRAEATRRVLER

SEQ ID NO: 5 - protein, 6 aa, synthetic construct
PGRRQH

SEQ ID NO: 6 - protein, 7 aa, synthetic construct
RRRGPKG

SEQ ID NO: 7 - protein, 7 aa, synthetic construct
RGERGEK

SEQ ID NO: 8 - protein, 10 aa, synthetic construct
RGLKGERGVK

SEQ ID NO: 9 - protein, 5 aa, synthetic construct
RWYHR

SEQ ID NO: 10 - DNA, 20 bp, synthetic construct
  source 1..20: mol_type = other DNA; note = amorce Gapdh F
catcaagaaggtggtgaagc

SEQ ID NO: 11 - DNA, 18 bp, synthetic construct
  source 1..18: mol_type = other DNA; note = amorce Gapdh R
accaccctgttgctgtag

SEQ ID NO: 12 - DNA, 20 bp, synthetic construct
  source 1..20: mol_type = other DNA; note = amorce Cyclophiline A F
ctaaggccaaccgtgaaaag

SEQ ID NO: 13 - DNA, 19 bp, synthetic construct
  source 1..19: mol_type = other DNA; note = amorce Cyclophiline A R
tacatggtcggggtcttga

SEQ ID NO: 14 - DNA, 20 bp, synthetic construct
  source 1..20: mol_type = other DNA; note = Amorce Act F
ggggagaaaggatttggcta

SEQ ID NO: 15 - DNA, 19 bp, synthetic construct
  source 1..19: mol_type = other DNA; note = amorce Act R
acatgcttgccatccagcc

SEQ ID NO: 16 - DNA, 20 bp, synthetic construct
  source 1..20: mol_type = other DNA; note = amorce Chtop F
cttaaagcagcgcctgggta

SEQ ID NO: 17 - DNA, 20 bp, synthetic construct
  source 1..20: mol_type = other DNA; note = amorce Chtop R
cacccctaagcagggttctg

SEQ ID NO: 18 - DNA, 21 bp, synthetic construct
  source 1..21: mol_type = other DNA; note = amorce Tfpi F
ttaatgctctgcccgaggaag

SEQ ID NO: 19 - DNA, 21 bp, synthetic construct
  source 1..21: mol_type = other DNA; note = amorce Tfpi R
aacctcggcagattccaggat

SEQ ID NO: 20 - DNA, 20 bp, synthetic construct
  source 1..20: mol_type = other DNA; note = amorce Adamts4 F
ggctgctgtaccgattacca

SEQ ID NO: 21 - DNA, 20 bp, synthetic construct
  source 1..20: mol_type = other DNA; note = amorce Adamts4 R
tctactcagcgaagcgaagc

SEQ ID NO: 22 - DNA, 20 bp, synthetic construct
  source 1..20: mol_type = other DNA; note = amorce Ccn1 F
gtgccgcctggtgaaagaga

SEQ ID NO: 23 - DNA, 24 bp, synthetic construct
  source 1..24: mol_type = other DNA; note = amorce Ccn1 R
gctgcatttcttgcccttttttag

SEQ ID NO: 24 - DNA, 22 bp, synthetic construct
  source 1..22: mol_type = other DNA; note = amorce Ndnf F
gaggaagataacaccccactgt

SEQ ID NO: 25 - DNA, 20 bp, synthetic construct
  source 1..20: mol_type = other DNA; note = amorce Ndnf F
cctgacccatctgcactgga

SEQ ID NO: 26 - DNA, 19 bp, synthetic construct
  source 1..19: mol_type = other DNA; note = amorce Hpse F
cggttctgacggactgctt

SEQ ID NO: 27 - DNA, 20 bp, synthetic construct
  source 1..20: mol_type = other DNA; note = amorce Hpse F
aaaacccataggaaaaggcg

SEQ ID NO: 28 - protein, 6 aa, synthetic construct
RLRARM

SEQ ID NO: 29 - protein, 8 aa, synthetic construct
LRKRLLRD

SEQ ID NO: 30 - protein, 6 aa, synthetic construct
PRRARV

SEQ ID NO: 31 - protein, 6 aa, synthetic construct
CRLYRK